European Patent Application EP 4 361 131 A1, published May 1, 2024. Title: OCT4 HIGH-SELECTIVITY ACTIVATOR. Applicant: IREGENE THERAPEUTICS LTD. The sequence listing filed with the application follows.

SEQUENCE LISTING (6 sequences)

SEQ ID NO: 1 - DNA, 20 bp, Artificial Sequence
  Chemically Synthesized
ccatgcattcaaactgaggt

SEQ ID NO: 2 - DNA, 21 bp, Artificial Sequence
  Chemically Synthesized
cctttgtgttcccaattcctt

SEQ ID NO: 3 - DNA, 22 bp, Artificial Sequence
  Chemically Synthesized
acctcagctacaaacaggtgaa

SEQ ID NO: 4 - DNA, 20 bp, Artificial Sequence
  Chemically Synthesized
aaaggctggggtaggtaggt

SEQ ID NO: 5 - DNA, 22 bp, Artificial Sequence
  Chemically Synthesized
ggccgaggactttgattgcaca

SEQ ID NO: 6 - DNA, 23 bp, Artificial Sequence
  Chemically Synthesized
gggcacgaaggctcatcattcaa